European Patent Application EP 4 631 572 A1, published October 15, 2025. Title: TMEM219 ANTIBODIES FOR MEDICAL USE. Applicant: Enthera S.r.l. Application EP. The sequence listing filed with the application follows.

SEQUENCE LISTING (180 sequences)

SEQ ID NO: 1 - protein, 5 aa, synthetic construct
SYAIS

SEQ ID NO: 2 - protein, 17 aa, synthetic construct
GIIPIFGTANYAQKFQG

SEQ ID NO: 3 - protein, 18 aa, synthetic construct
GDIAAAGRKGLPIYYMDV

SEQ ID NO: 4 - protein, 214 aa, synthetic construct
QAVLTQPPSVSVSPGQTASITCSGDKLGNKNAYWYQQKPGQSPVLVMYQSTRRPSGIPERFSASNSGNTATLTISGTQAMDEADYYCQAWDSSSGWEVFGGGTKLTVLGQPKAAPSVTLFPPSSEELQANKATLVCLISDFYPGAVTVAWKADSSPVKAGVETTTPSKQSNNKYAASSYLSLTPEQWKSHRSYSCQVTHEGSTVEKTVAPTECS

SEQ ID NO: 5 - protein, 17 aa, synthetic construct
WISAYNGNTNYAQKLQG

SEQ ID NO: 6 - protein, 9 aa, synthetic construct
WGRWLAHDY

SEQ ID NO: 7 - protein, 12 aa, synthetic construct
PSGYYIYDAFDI

SEQ ID NO: 8 - protein, 5 aa, synthetic construct
SYGIS

SEQ ID NO: 9 - protein, 8 aa, synthetic construct
DLGWPDDY

SEQ ID NO: 10 - protein, 5 aa, synthetic construct
DYGMS

SEQ ID NO: 11 - protein, 17 aa, synthetic construct
GINWNGGSTGYADSVKG

SEQ ID NO: 12 - protein, 16 aa, synthetic construct
DRLRYCSSTSCYIPDY

SEQ ID NO: 13 - protein, 19 aa, synthetic construct
VGSTYDFWSGAYYYYGMDV

SEQ ID NO: 14 - protein, 11 aa, synthetic construct
QASQDISNYLN

SEQ ID NO: 15 - protein, 7 aa, synthetic construct
AASSLQS

SEQ ID NO: 16 - protein, 8 aa, synthetic construct
QQSYSTPT

SEQ ID NO: 17 - protein, 11 aa, synthetic construct
SGDKLGNKNAY

SEQ ID NO: 18 - protein, 7 aa, synthetic construct
QSTRRPS

SEQ ID NO: 19 - protein, 11 aa, synthetic construct
QAWDSSSGWEV

SEQ ID NO: 20 - protein, 12 aa, synthetic construct
GASQSVSSSYLA

SEQ ID NO: 21 - protein, 7 aa, synthetic construct
DASSRAT

SEQ ID NO: 22 - protein, 9 aa, synthetic construct
HQYNNWPRT

SEQ ID NO: 23 - protein, 13 aa, synthetic construct
SGSSSNIGSNYVY

SEQ ID NO: 24 - protein, 7 aa, synthetic construct
RNNQRPS

SEQ ID NO: 25 - protein, 11 aa, synthetic construct
AAWDDSLNGVV

SEQ ID NO: 26 - protein, 17 aa, synthetic construct
KSSQSVLDSSNNKNYVA

SEQ ID NO: 27 - protein, 7 aa, synthetic construct
WASTRES

SEQ ID NO: 28 - protein, 9 aa, synthetic construct
QQYYTTRWT

SEQ ID NO: 29 - protein, 11 aa, synthetic construct
RASQGIRNDLG

SEQ ID NO: 30 - protein, 7 aa, synthetic construct
DASNLET

SEQ ID NO: 31 - protein, 9 aa, synthetic construct
QQYDNLPLT

SEQ ID NO: 32 - protein, 127 aa, synthetic construct
QVQLVQSGAEVKRPGSSVKVSCKASGGTFSSYAISWVRQAPGQGLEWMGGIIPIFGTANYAQKFQGRVTITADESTSTAYMELSNLRSEDTAVYYCARGDIAAAGRKGLPIYYMDVWGKGTTVTVSS

SEQ ID NO: 33 - protein, 118 aa, synthetic construct
QIQLVQSGAEVKKPGASVKVSCKASGYTFTSYGISWVRQAPGQGLEWMGWISAYNGNTNYAQKLQGRVTMTTDTSTSTAYMELRSLRSDDTAVYYCARWGRWLAHDYWGQGTLVTVSS

SEQ ID NO: 34 - protein, 121 aa, synthetic construct
QMQLVQSGAEVKKPGSSVKVSCKASGGTFSSYAISWVRQAPGQGLEWMGGIIPIFGTANYAQKFQGRVTITADESTSTAYMELSSLRSEDTAVYYCASPSGYYIYDAFDIWGQGTMVTVSS

SEQ ID NO: 35 - protein, 117 aa, synthetic construct
QVQLVQSGAEVKKPGASVKVSCKASGYTFTSYGISWVRQAPGQGLEWMGWISAYNGNTNYAQKLQGRVTMTTDTSTSTAYMELRSLRSDDTAVYYCARDLGWPDDYWGQGTLVTVSS

SEQ ID NO: 36 - protein, 125 aa, synthetic construct
EVQLLESGGGVVRPGGSLRLSCAASGFTFDDYGMSWVRQAPGKGLEWVSGINWNGGSTGYADSVKGRFTISRDNSKNTLYLQMNSLRAEDTAAYYCAKDRLRYCSSTSCYIPDYWGQGTLVTVSS

SEQ ID NO: 37 - protein, 128 aa, synthetic construct
QVQLVQSGAEVKKPGASVKVSCKASGYTFTSYGISWVRQAPGQGLEWMGWISAYNGNTNYAQKLQGRVTMTTDTSTSTAYMELRSLRSDDTAVYYCARVGSTYDFWSGAYYYYGMDVWGQGTTVTVSS

SEQ ID NO: 38 - protein, 106 aa, synthetic construct
DIQMTQSPSSLSASVGDRVTITCQASQDISNYLNWYQQKPGKAPKLLIYAASSLQSGVPSRFSGSGSGTDFTLTISSLQPEDFATYYCQQSYSTPTFGQGTKLEIK

SEQ ID NO: 39 - protein, 108 aa, synthetic construct
QAVLTQPPSVSVSPGQTASITCSGDKLGNKNAYWYQQKPGQSPVLVMYQSTRRPSGIPERFSASNSGNTATLTISGTQAMDEADYYCQAWDSSSGWEVFGGGTKLTVL

SEQ ID NO: 40 - protein, 108 aa, synthetic construct
ETTLTQSPATLSLSPGERATLSCGASQSVSSSYLAWYQQKPGLAPRLLIYDASSRATGIPDRFSGSGSGTDFTLTISRLEPEDFAVYYCHQYNNWPRTFGQGTKVEIK

SEQ ID NO: 41 - protein, 110 aa, synthetic construct
QPVLTQPPSASGTPGQRVTISCSGSSSNIGSNYVYWYQQLPGTAPKLLIYRNNQRPSGVPDRFSGSKSGTSASLAISGLRSEDEADYYCAAWDDSLNGVVFGGGTKLTVL

SEQ ID NO: 42 - protein, 113 aa, synthetic construct
DIQMTQSPDSLAVSLGERATINCKSSQSVLDSSNNKNYVAWFQQKPGQPPKLLIYWASTRESGVPDRFSGSGSGTDFTLTISSLQAEDVAVYYCQQYYTTRWTFGQGTKVEIK

SEQ ID NO: 43 - protein, 107 aa, synthetic construct
DIVMTQSPSSLSASVGDRVTITCRASQGIRNDLGWYQQKPGKAPKLLIYDASNLETGVPSRFSGSGSGTDFTFTISSLQPEDIATYYCQQYDNLPLTFGGGTKVEIK

SEQ ID NO: 44 - protein, 381 aa, synthetic construct
CAGGTCCAGCTGGTACAGTCTGGGGCTGAGGTGAAGAGGCCTGGGTCCTCGGTGAAGGTCTCCTGCAAGGCTTCTGGAGGCACCTTCAGCAGCTATGCTATCAGCTGGGTGCGACAGGCCCCTGGACAAGGGCTTGAGTGGATGGGAGGGATCATCCCTATCTTTGGTACAGCAAACTACGCACAGAAGTTCCAGGGCAGAGTCACGATTACCGCGGACGAATCCACGAGCACAGCCTACATGGAGCTGAGCAACCTGAGATCTGAGGACACGGCCGTGTATTACTGTGCGAGAGGGGATATAGCAGCAGCTGGTAGGAAAGGACTGCCCATCTACTACATGGACGTCTGGGGCAAAGGGACCACGGTCACCGTCTCCTCA

SEQ ID NO: 45 - DNA, 354 bp, synthetic construct
  source 1..354: mol_type = other DNA
caaatccagctggtacagtctggggctgaggtgaagaagcctggggcctcagtgaaggtctcctgcaaggcttctggttacacctttaccagctacggtatcagctgggtgcgacaggcccctggacaagggcttgagtggatgggatggatcagcgcttacaatggtaacacaaactatgcacagaagctccagggcagagtcaccatgaccacagacacatccacgagcacagcctacatggagctgaggagcctgagatctgacgacacggccgtgtattactgtgcgaggtggggtaggtggctggctcatgactactggggccagggaaccctggtcaccgtctcctca

SEQ ID NO: 46 - DNA, 363 bp, synthetic construct
  source 1..363: mol_type = other DNA
cagatgcagctggtgcagtctggggctgaggtgaagaagcctgggtcctcggtgaaggtctcctgcaaggcttctggaggcaccttcagcagctatgctatcagctgggtgcgacaggcccctggacaagggcttgagtggatgggagggatcatccctatctttggtacagcaaactacgcacagaagttccagggcagagtcacgattaccgcggacgaatccacgagcacagcctacatggagctgagcagcctgagatctgaggacacggccgtgtattactgtgcgagcccaagtggttattatatttatgatgcttttgatatctggggccaagggacaatggtcaccgtctcttca

SEQ ID NO: 47 - DNA, 351 bp, synthetic construct
  source 1..351: mol_type = other DNA
caggtccagctggtgcagtctggagctgaggtgaagaagcctggggcctcagtgaaggtctcctgcaaggcttctggttacacctttaccagctatggtatcagctgggtgcgacaggcccctggacaagggcttgagtggatgggatggatcagcgcttacaatggtaacacaaactatgcacagaagctccagggcagagtcaccatgaccacagacacatccacgagcacagcctacatggagctgaggagcctgagatctgacgacacggccgtgtattactgtgcgagagatctcggctggccagatgactactggggccagggaaccctggtcaccgtctcctca

SEQ ID NO: 48 - DNA, 375 bp, synthetic construct
  source 1..375: mol_type = other DNA
gaagtgcagttgttggagtctgggggaggtgtggtacggcctggggggtccctgagactctcctgtgcagcctctggattcacctttgatgattatggcatgagctgggtccgccaagctccagggaaggggctggagtgggtctctggtattaattggaatggtggtagcacaggttatgcagactccgtgaagggccgattcaccatctccagagacaattccaagaacacgctgtatctgcaaatgaacagcctgagagctgaggacacggctgcgtattactgtgcgaaagatcgactaagatattgtagtagtaccagctgctatatccctgactactggggccagggaaccctggtcaccgtctcctca

SEQ ID NO: 49 - DNA, 384 bp, synthetic construct
  source 1..384: mol_type = other DNA
caggtgcagctggtgcagtctggagctgaggtgaagaagcctggggcctcagtgaaggtctcctgcaaggcttctggttacacctttaccagctatggtatcagctgggtgcgacaggcccctggacaagggcttgagtggatgggatggatcagcgcttacaatggtaacacaaactatgcacagaagctccagggcagagtcaccatgaccacagacacatccacgagcacagcctacatggagctgaggagcctgagatctgacgacacggccgtgtattactgtgcgagagtagggagcacttacgatttttggagtggcgcctactactactacggtatggacgtctggggccaagggaccacggtcaccgtctcctca

SEQ ID NO: 50 - DNA, 318 bp, synthetic construct
  source 1..318: mol_type = other DNA
gacatccagatgacccagtctccatcctccctgtctgcatctgtaggagacagagtcaccatcacttgccaggcgagtcaggacattagcaactacttaaattggtatcagcagaaaccagggaaagcccctaagctcctgatctatgctgcatccagtttgcaaagtggggtcccatcaaggttcagtggcagtggatctgggacagatttcactctcaccatcagcagtctgcaacctgaagattttgcaacttactactgtcaacagagttacagtacccctacttttggccaggggaccaagctggagatcaaa

SEQ ID NO: 51 - DNA, 324 bp, synthetic construct
  source 1..324: mol_type = other DNA
caggcagtgctgactcagccaccctcagtgtccgtgtccccaggacagacagccagcatcacctgctctggagataaattgggaaataaaaatgcttattggtatcagcagaagccaggccagtcccctgtactggtcatgtatcaaagtaccagacggccctcagggatccctgagcgattctctgcctccaactctgggaacacagccactctgaccatcagcgggacccaggctatggatgaggctgactattactgtcaggcgtgggacagcagtagtggatgggaggtattcggcggagggaccaagctgaccgtccta

SEQ ID NO: 52 - DNA, 324 bp, synthetic construct
  source 1..324: mol_type = other DNA
gaaacgacactcacgcagtctccagccaccctgtctttgtctccaggggaaagagccaccctctcctgcggggccagtcagagtgttagcagcagctacttagcctggtaccagcagaaacctggcctggcgcccaggctcctcatctatgatgcatccagcagggccactggcatcccagacaggttcagtggcagtgggtctgggacagacttcactctcaccatcagcagactggagcctgaagattttgcagtttattactgtcaccagtataataactggcctaggacgttcggccaagggaccaaggtggaaatcaaa

SEQ ID NO: 53 - DNA, 330 bp, synthetic construct
  source 1..330: mol_type = other DNA
cagcctgtgctgactcagccaccctcagcgtctgggacccccgggcagagggtcaccatctcttgttctggaagcagctccaacatcggaagtaattatgtatactggtaccagcagctcccaggaacggcccccaaactcctcatctataggaataatcagcggccctcaggggtccctgaccgattctctggctccaagtctggcacctcagcctccctggccatcagtgggctccggtccgaggatgaggctgattattattgtgcagcatgggatgacagcctgaatggtgtggtattcggcggagggaccaagctgaccgtccta

SEQ ID NO: 54 - DNA, 339 bp, synthetic construct
  source 1..339: mol_type = other DNA
gacatccagatgacccagtctccggactccctggctgtgtctctgggcgagagggccaccatcaactgcaagtccagccagagtgttttggacagctccaacaataaaaattatgtcgcttggttccagcagaaaccaggacagcctcctaagctgctcatttactgggcctctacccgggaatccggggtccctgaccgattcagtggcagcggttctgggacagatttcactctcaccatcagcagcctgcaggctgaagatgtggcagtttattactgtcagcaatattatactactcggtggacgttcggccaagggaccaaggtggaaatcaaa

SEQ ID NO: 55 - DNA, 321 bp, synthetic construct
  source 1..321: mol_type = other DNA
gacatcgtgatgacccagtctccatcctccctgtctgcatctgtaggagacagagtcaccatcacttgccgggcaagtcagggcattagaaatgatttaggctggtatcagcaaaaaccagggaaagcccctaaactcctgatctacgatgcatccaatttggaaacaggggtcccatcaaggttcagtggaagtggatctgggacagattttactttcaccatcagcagcctgcagcctgaagatattgcaacatattactgtcaacagtatgataacctcccgctcactttcggcggagggaccaaggtggagatcaaa

SEQ ID NO: 56 - protein, 8 aa, synthetic construct
GFTFSRHG

SEQ ID NO: 57 - protein, 8 aa, synthetic construct
IWYDGRNK

SEQ ID NO: 58 - protein, 17 aa, synthetic construct
AREGITMVRGVIPLFDY

SEQ ID NO: 59 - protein, 8 aa, synthetic construct
GFTFSRYG

SEQ ID NO: 60 - protein, 8 aa, synthetic construct
IWYDGSYK

SEQ ID NO: 61 - protein, 13 aa, synthetic construct
ARFGILTGYYFDY

SEQ ID NO: 62 - protein, 8 aa, synthetic construct
GFTFSSYA

SEQ ID NO: 63 - protein, 8 aa, synthetic construct
ISGSGYST

SEQ ID NO: 64 - protein, 13 aa, synthetic construct
AKGKVGPTYAFDL

SEQ ID NO: 65 - protein, 8 aa, synthetic construct
GFTFSSYG

SEQ ID NO: 66 - protein, 8 aa, synthetic construct
IWYDGSNK

SEQ ID NO: 67 - protein, 9 aa, synthetic construct
AREGRGMDV

SEQ ID NO: 68 - protein, 8 aa, synthetic construct
GFTFSTYG

SEQ ID NO: 69 - protein, 8 aa, synthetic construct
IWYDGYNK

SEQ ID NO: 70 - protein, 13 aa, synthetic construct
EGWFGKLLSALDI

SEQ ID NO: 71 - protein, 7 aa, synthetic construct
SGHSSYA

SEQ ID NO: 72 - protein, 7 aa, synthetic construct
LNSDGSH

SEQ ID NO: 73 - protein, 9 aa, synthetic construct
QTWGTGMLC

SEQ ID NO: 74 - protein, 9 aa, synthetic construct
QTWGTGMLF

SEQ ID NO: 75 - protein, 9 aa, synthetic construct
QTWGTGMLW

SEQ ID NO: 76 - protein, 8 aa, synthetic construct
QTWGTGCC

SEQ ID NO: 77 - protein, 9 aa, synthetic construct
SGSVSTSYN

SEQ ID NO: 78 - skipped

SEQ ID NO: 79 - protein, 9 aa, synthetic construct
VLYMGSGII

SEQ ID NO: 80 - protein, 9 aa, synthetic construct
SGSVSTSYY

SEQ ID NO: 81 - protein, 10 aa, synthetic construct
VLYMGSGTCC

SEQ ID NO: 82 - protein, 7 aa, synthetic construct
SGHSSYI

SEQ ID NO: 83 - protein, 7 aa, synthetic construct
LEGSGSY

SEQ ID NO: 84 - protein, 11 aa, synthetic construct
ETWDSNTPHAV

SEQ ID NO: 85 - protein, 6 aa, synthetic construct
QGIRND

SEQ ID NO: 86 - skipped

SEQ ID NO: 87 - protein, 9 aa, synthetic construct
LQDYNYPFT

SEQ ID NO: 88 - protein, 124 aa, synthetic construct
QVQLVESGGGVVQPGRSLRLSCAASGFTFSRHGMHWVRQAPGKGLEWVAVIWYDGRNKYYADSVKGRFTISRDNSKNTLYLQMNSLRVEDTAVYYCAREGITMVRGVIPLFDYWGQGTLVTVSS

SEQ ID NO: 89 - protein, 124 aa, synthetic construct; identical to SEQ ID NO: 88

SEQ ID NO: 90 - protein, 124 aa, synthetic construct; identical to SEQ ID NO: 88

SEQ ID NO: 91 - protein, 120 aa, synthetic construct
QVQLVESGGGVVQPGRSLRLSCAASGFTFSRYGMHWVRQAPGKGLEWVAVIWYDGSYKYYADSIKGRFTVSRDNSKNTLYLQMNSLRAEDTALYYCARFGILTGYYFDYWGQGTLVTVSS

SEQ ID NO: 92 - protein, 124 aa, synthetic construct; identical to SEQ ID NO: 88

SEQ ID NO: 93 - protein, 120 aa, synthetic construct
EVQLLESGGGLVQPGGSLRLSCAASGFTFSSYAMSWVRQAPGEGLEWVSGISGSGYSTYSADSVKGRFTIFKDNSKNTLYLQINSLRAEDTAVYYCAKGKVGPTYAFDLWGQGTMVTVSS

SEQ ID NO: 94 - protein, 116 aa, synthetic construct
QVQLVESGGGVVQPGRSLRLSCAASGFTFSSYGMHWVRQAPGKGLEWVAVIWYDGSNKYYADSVKGRFTISRDNSKNTLYLQMNSLRAEDTAVYYCAREGRGMDVWGQGTTVTVSS

SEQ ID NO: 95 - protein, 122 aa, synthetic construct
QVQLVESGGGVVQPGRSLRLSCAASGFTFSTYGIHWVRQAPGKGLEWVAVIWYDGYNKYYVDSVKGRFTISRDNSENTVYLQMNSLRTEDTAVYYCAREGWFGKLLSALDIWGQGTMVTVSS

SEQ ID NO: 96 - protein, 112 aa, synthetic construct
QFVLTQSPSASASLGASVKLTCTLSSGHSSYAIAWHHQQPEKGPRYLMKLNSDGSHSKGDGIPDRFSGSSSGAERYLTISSLQSEDEADYYCQTWGTGMLCFGGGTQLTALR

SEQ ID NO: 97 - protein, 111 aa, synthetic construct
QFVLTQSPSASASLGASVKLTCTLSSGHSSYAIAWHHQQPEKGPRYLMKLNSDGSHSKGDGIPDRFSGSSSGAERYLTISSLQSEDEADYYCQTWGTGMLFGGGTQLTALR

SEQ ID NO: 98 - protein, 112 aa, synthetic construct
QFVLTQSPSASASLGASVKLTCTLSSGHSSYAIAWHHQQPEKGPRYLMKLNSDGSHSKGDGIPDRFSGSSSGAERYLTISSLQSEDEADYYCQTWGTGMLWFGGGTQLTALR

SEQ ID NO: 99 - protein, 111 aa, synthetic construct
QVVLTQSPPASASLGASVKLTCTLSSGHSSYAIAWHQQQPEKGPRYLMKLNSDGSHSKGDGIPDRFSGSSSGAERYLTISSLQSEDEADYYCQTWGTGCCFGGGTQLTALR

SEQ ID NO: 100 - protein, 109 aa, synthetic construct
QTVVTQESSFSVSPGGTVTLTCGLSSGSVSTSYNPSWYQQTPGQAPRTLIYSTNTRSSGVPDRFSGSILGNKAALTITGAQADDESDYYCVLYMGSGIIFGSGTKVTVL

SEQ ID NO: 101 - protein, 111 aa, synthetic construct
QTVVTQEPSFSVSPGGTVTLTCGLSSGSVSTSYYPSWYQQTPGQAPRTLIYSTNTRSSGVPERFSGSILGNKAALTITGAQADDESDYYCVLYMGSGTCCFGGGTQLTALR

SEQ ID NO: 102 - protein, 113 aa, synthetic construct
QPVLTQSSSASASLGSSVKLTCTLSSGHSSYIIAWHQQQPGKAPRYLMKLEGSGSYNKGSGVPDRFSGSSSGADRYLTISNLQFEDEADYYCETWDSNTPHAVFGGGTQLTAL

SEQ ID NO: 103 - protein, 107 aa, synthetic construct
VIQMTQSPSSLSASVGDRVTITCRASQGIRNDLGWYLQKPGKAPELLIYPASSLQSGVPSRFSGSGSGTDFTLTISSLQPEDFATYYCLQDYNYPFTFGQGTKLEIK

SEQ ID NO: 104 - protein, 372 aa, synthetic construct
CAGGTCCAACTCGTCGAGAGCGGAGGAGGAGTCGTCCAACCCGGAAGGAGCTTGCGGCTATCATGCGCGGCATCCGGCTTCACATTTTCCCGGCACGGGATGCACTGGGTCAGGCAAGCACCCGGCAAGGGGCTAGAATGGGTCGCGGTCATCTGGTATGATGGAAGGAACAAATACTATGCCGACTCAGTCAAGGGGCGATTTACAATTTCGCGAGACAACTCCAAGAATACGCTATACCTGCAAATGAACTCGCTGAGGGTCGAGGACACGGCGGTTTATTACTGCGCGAGGGAGGGGATAACTATGGTCAGAGGAGTCATTCCGCTATTTGACTATTGGGGGCAGGGTACCTTAGTCACGGTCTCGAGC

SEQ ID NO: 105 - DNA, 372 bp, synthetic construct
  source 1..372: mol_type = other DNA
caggtccaactcgtcgagagcggaggaggagtcgtccaacccggaaggagcttgcggctatcatgcgcggcatccggcttcacattttcccggcacgggatgcactgggtcaggcaagcacccggcaaggggctagaatgggtcgcggtcatctggtatgatggaaggaacaaatactatgccgactcagtcaaggggcgatttacaatttcgcgagacaactccaagaatacgctatacctgcaaatgaactcgctgagggtcgaggacacggcggtttattactgcgcgagggaggggataactatggtcagaggagtcattccgctatttgactattgggggcagggtaccttagtcacggtctcgagc

SEQ ID NO: 106 - DNA, 372 bp, synthetic construct; identical to SEQ ID NO: 105
  source 1..372: mol_type = other DNA

SEQ ID NO: 107 - DNA, 360 bp, synthetic construct
  source 1..360: mol_type = other DNA
caggtccaactcgttgaatccggggggggagtcgtccaaccggggagaagcctgcggctaagctgcgcggcttcgggattcacattctctcgatacgggatgcactgggtcaggcaagcaccggggaagggcttggaatgggtcgccgtcatatggtacgacggatcatataaatattatgctgactctataaaggggcgattcacggttagccgagacaactccaaaaacacgctatacctgcaaatgaactcactgcgagctgaagatacggcgctatattattgcgcccgattcggaatcctgaccggatattattttgactactgggggcagggtaccctagtcacggtctcgagc

SEQ ID NO: 108 - DNA, 372 bp, synthetic construct; identical to SEQ ID NO: 105
  source 1..372: mol_type = other DNA

SEQ ID NO: 109 - DNA, 360 bp, synthetic construct
  source 1..360: mol_type = other DNA
gaagtccaactgctggaatcgggcggggggctggtccaacccggaggatcattgaggctatcatgcgccgcttccggctttacatttagctcatacgcaatgtcatgggtccgacaagctccgggggagggactggaatgggtctctgggatttcgggctctggatactccacatatagcgcggactcagtcaaggggagattcacgatttttaaggataactccaagaatacattatatctgcaaataaactcgctgagggcggaggataccgccgtttattactgcgccaaagggaaagtcgggccaacttacgcattcgacctatgggggcagggtaccatggtcacggtctcgagc

SEQ ID NO: 110 - DNA, 348 bp, synthetic construct
  source 1..348: mol_type = other DNA
caagtgcaactcgtggaatcgggcggaggggtggtgcaaccgggaagatcactgcgactatcatgcgccgcatcgggatttacatttagcagctacgggatgcactgggtccgccaagcacccggaaaagggctggaatgggtcgcggtgatttggtacgatggctcgaataaatactatgctgactcggtgaagggccgattcacaatctcgcgggacaactccaaaaacacactatatctgcaaatgaactcactgcgggcggaggataccgcggtatattactgcgcgagggaggggcgcggaatggatgtatgggggcagggtaccacggtgaccgtctcgagc

SEQ ID NO: 111 - DNA, 366 bp, synthetic construct
  source 1..366: mol_type = other DNA
caggtgcagctggtggagtctgggggaggcgtggtccagcctgggaggtccctgagactctcctgtgcagcatctggattcaccttcagtacctatggcatacactgggtccgccaggctccaggcaaggggctggagtgggtggcagttatatggtatgatggatataataaatactatgtagactccgtgaagggccgattcaccatctccagagacaattccgagaacacggtgtatctgcagatgaacagcctgagaaccgaggacacggctgtttattactgtgcgagagaaggatggttcgggaaattattatccgctcttgatatctggggccaagggacaatggtcaccgtctcttca

SEQ ID NO: 112 - DNA, 408 bp, synthetic construct
  source 1..408: mol_type = other DNA
gcggccgccatgaattttggactgaggctgattttcctggtgctgaccctgaaaggcgtccagtgtcaatttgtgctgacgcaatcgccatcggctagtgcatcactgggggcgagcgttaaattgacatgcacgctatcgagcggacactcatcatatgccattgcatggcaccaccaacaaccggaaaaggggccacgatatctaatgaagctgaactctgacggatcgcattcgaaaggggatgggattcccgaccgattctcgggaagcagcagcggagctgaaagatatttaacgatatcatcgctgcaatcggaggatgaagctgactactactgccaaacttggggaacggggatgctatgcttcggaggaggcacacaattgacggcccttggacaaccg

SEQ ID NO: 113 - DNA, 405 bp, synthetic construct
  source 1..405: mol_type = other DNA
gcggccgccatgaattttggactgaggctgattttcctggtgctgaccctgaaaggcgtccagtgtcaatttgtactgacgcaaagcccaagcgcgagcgcatcgctgggagcatccgtcaagctcacatgcacgctatcatcgggccattcaagctatgccatagcatggcatcaccaacaaccggagaagggacctcgatatctgatgaagctgaatagcgacggctcccactcaaagggggacggaatcccggatagattttcgggctcatcaagcggagcggagcgatatctcacgatctctagcctgcaaagcgaggatgaggccgactactactgccaaacatgggggacgggaatgctattcggaggaggcacgcaactgacggcgctggggcaacca

SEQ ID NO: 114 - DNA, 408 bp, synthetic construct
  source 1..408: mol_type = other DNA
gcggccgccatgaattttggactgaggctgattttcctggtgctgaccctgaaaggcgtccagtgtcaatttgtgctgacgcaatcaccatcggcttcggcgagcctgggggcatctgtcaagctgacatgcacgctgagctccgggcattcatcatatgccatcgcatggcatcaccaacaacccgagaagggaccacgatatctcatgaagctaaactccgacggatcgcattcgaagggggatggaatacccgaccgattttcgggatcatcgagcggggcggagagatatttgacgatctcctctctgcaaagcgaggacgaggcggactactattgccaaacctggggcacgggaatgctatggtttggaggaggcacacaactgacggcgctgggccaaccg

SEQ ID NO: 115 - DNA, 405 bp, synthetic construct
  source 1..405: mol_type = other DNA
gcggccgccatgaattttggactgaggctgattttcctggtgctgaccctgaaaggcgtccagtgtcaagtagtcctgactcaaagccccccggcgagcgcatcattgggggcgagcgtcaagctgacatgcacgctatcgagcgggcactctagctacgcgatagcatggcaccaacaacaaccggaaaagggaccccgatacttgatgaaattaaatagcgacggatcgcactctaagggagacggaatacctgatagatttagcgggagctcatcgggggcggagagatacttgacgattagctcactgcaatcggaggatgaggcggactactattgccaaacatgggggacgggatgctgcttcggaggaggcacgcaactgaccgcattgggacaacca

SEQ ID NO: 116 - DNA, 402 bp, synthetic construct
  source 1..402: mol_type = other DNA
gcggccgccatgaattttggactgaggctgattttcctggtgctgaccctgaaaggcgtccagtgtcaaaccgtggtgacacaagaatcaagttttagcgtatcgccgggagggacggtgacgctgacctgcgggctatcatctggatcggtatcaacatcctacaatccgagctggtatcaacaaacgcccggacaagcgccacgaaccctgatatattcgacaaatacccgatcatctggggtgccggatagattttccggctcgattctgggaaacaaggctgcgctgacgataaccggagctcaagccgacgatgagagcgattattattgcgtgctatacatggggagcgggattatattcggatctggaacgaaagtcacggtgctaggacaaccg

SEQ ID NO: 117 - DNA, 405 bp, synthetic construct
  source 1..405: mol_type = other DNA
gcggccgccatgaattttggactgaggctgattttcctggtgctgaccctgaaaggcgtccagtgtcaaacggtcgtcacgcaagagccatccttctcggtctcgccgggggggacggtcacactgacatgcgggctgagctcgggatcggtctcaacgagctactacccgagctggtatcaacaaacaccggggcaagcaccgcggacgctgatatattccacaaatacacggagctccggtgtcccggagagattctcgggatcaatactggggaacaaggcggctctgacgataaccggagcccaagcggatgacgaatcggactattactgcgtcctatacatgggctccggcacatgctgctttggaggaggcacacaactgacggcgctgggacaacct

SEQ ID NO: 118 - DNA, 414 bp, synthetic construct
  source 1..414: mol_type = other DNA
gcggccgccatgaattttggactgaggctgattttcctggtgctgaccctgaaaggcgtccagtgtcagccggttttgacgcaatctagcagcgcatccgctagtcttggaagctccgtgaagctgacatgcacactatcatcggggcattcctcctacataattgcatggcatcaacaacaacccggcaaggccccgagatacttaatgaaactggaaggatcgggatcatataacaaaggatcgggggtgccggatagatttagcggatctagctctggggctgaccgatacctgacgatctctaatctgcaatttgaggacgaggccgattactactgcgaaacatgggatagcaacaccccacacgcggtatttggaggaggcacccaattgaccgcgctaggccaacca

SEQ ID NO: 119 - DNA, 321 bp, synthetic construct
  source 1..321: mol_type = other DNA
gtcatccagatgacccagtctccatcctccctgtctgcatctgtaggagacagagtcaccatcacttgccgggcaagtcagggcattagaaatgatttaggctggtatctgcagaaaccagggaaagcccctgagctcctgatctatcctgcatccagtttacaaagtggggtcccgtcaaggttcagcggcagtggatctggcacagatttcactctcaccatcagcagcctgcagcctgaagattttgcaacttattactgtctacaagattacaattacccgttcacttttggccaggggaccaagctggagatcaaa

SEQ ID NO: 120 - protein, 327 aa, synthetic construct
ASTKGPSVFPLAPCSRSTSESTAALGCLVKDYFPEPVTVSWNSGALTSGVHTFPAVLQSSGLYSLSSVVTVPSSSLGTKTYTCNVDHKPSNTKVDKRVESKYGPPCPPCPAPEFEGGPSVFLFPPKPKDTLMISRTPEVTCVVVDVSQEDPEVQFNWYVDGVEVHNAKTKPREEQFNSTYRVVSVLTVLHQDWLNGKEYKCKVSNKGLPSSIEKTISKAKGQPREPQVYTLPPSQEEMTKNQVSLTCLVKGFYPSDIAVEWESNGQPENNYKTTPPVLDSDGSFFLYSRLTVDKSRWQEGNVFSCSVMHEALHNHYTQKSLSLSLGK

SEQ ID NO: 121 - protein, 326 aa, synthetic construct
ASTKGPSVFPLAPCSRSTSESTAALGCLVKDYFPEPVTVSWNSGALTSGVHTFPAVLQSSGLYSLSSVVTVPSSNFGTQTYTCNVDHKPSNTKVDKTVERKCCVECPPCPAPPVAGPSVFLFPPKPKDTLMISRTPEVTCVVVDVSHEDPEVQFNWYVDGVEVHNAKTKPREEQFNSTFRVVSVLTVVHQDWLNGKEYKCKVSNKGLPAPIEKTISKTKGQPREPQVYTLPPSREEMTKNQVSLTCLVKGFYPSDISVEWESNGQPENNYKTTPPMLDSDGSFFLYSKLTVDKSRWQQGNVFSCSVMHEALHNHYTQKSLSLSPGK

SEQ ID NO: 122 - protein, 106 aa, synthetic construct
GQPKANPTVTLFPPSSEELQANKATLVCLISDFYPGAVTVAWKADGSPVKAGVETTKPSKQSNNKYAASSYLSLTPEQWKSHRSYSCQVTHEGSTVEKTVAPTECS

SEQ ID NO: 123 - protein, 106 aa, synthetic construct
GQPKAAPSVTLFPPSSEELQANKATLVCLISDFYPGAVTVAWKADSSPVKAGVETTTPSKQSNNKYAASSYLSLTPEQWKSHRSYSCQVTHEGSTVEKTVAPTECS

SEQ ID NO: 124 - protein, 107 aa, synthetic construct [sequence omitted]

SEQ ID NO: 125 - protein, 445 aa, synthetic construct
QIQLVQSGAEVKKPGASVKVSCKASGYTFTSYGISWVRQAPGQGLEWMGWISAYNGNTNYAQKLQGRVTMTTDTSTSTAYMELRSLRSDDTAVYYCARWGRWLAHDYWGQGTLVTVSSASTKGPSVFPLAPCSRSTSESTAALGCLVKDYFPEPVTVSWNSGALTSGVHTFPAVLQSSGLYSLSSVVTVPSSSLGTKTYTCNVDHKPSNTKVDKRVESKYGPPCPPCPAPEFEGGPSVFLFPPKPKDTLMISRTPEVTCVVVDVSQEDPEVQFNWYVDGVEVHNAKTKPREEQFNSTYRVVSVLTVLHQDWLNGKEYKCKVSNKGLPSSIEKTISKAKGQPREPQVYTLPPSQEEMTKNQVSLTCLVKGFYPSDIAVEWESNGQPENNYKTTPPVLDSDGSFFLYSRLTVDKSRWQEGNVFSCSVMHEALHNHYTQKSLSLSLGK

SEQ ID NO: 126 - protein, 444 aa, synthetic construct
QIQLVQSGAEVKKPGASVKVSCKASGYTFTSYGISWVRQAPGQGLEWMGWISAYNGNTNYAQKLQGRVTMTTDTSTSTAYMELRSLRSDDTAVYYCARWGRWLAHDYWGQGTLVTVSSASTKGPSVFPLAPCSRSTSESTAALGCLVKDYFPEPVTVSWNSGALTSGVHTFPAVLQSSGLYSLSSVVTVPSSSLGTKTYTCNVDHKPSNTKVDKRVESKYGPPCPPCPAPEFEGGPSVFLFPPKPKDTLMISRTPEVTCVVVDVSQEDPEVQFNWYVDGVEVHNAKTKPREEQFNSTYRVVSVLTVLHQDWLNGKEYKCKVSNKGLPSSIEKTISKAKGQPREPQVYTLPPSQEEMTKNQVSLTCLVKGFYPSDIAVEWESNGQPENNYKTTPPVLDSDGSFFLYSRLTVDKSRWQEGNVFSCSVMHEALHNHYTQKSLSLSLG

SEQ ID NO: 127 - protein, 30 aa, synthetic construct
QIQLVQSGAEVKKPGASVKVSCKASGYTFT

SEQ ID NO: 128 - protein, 14 aa, synthetic construct
WVRQAPGQGLEWMG

SEQ ID NO: 129 - protein, 32 aa, synthetic construct
RVTMTTDTSTSTAYMELRSLRSDDTAVYYCAR

SEQ ID NO: 130 - protein, 11 aa, synthetic construct
WGQGTLVTVSS

SEQ ID NO: 131 - protein, 25 aa, synthetic construct
QIQLVQSGAEVKKPGASVKVSCKAS

SEQ ID NO: 132 - protein, 8 aa, synthetic construct
GYTFTSYG

SEQ ID NO: 133 - protein, 17 aa, synthetic construct
ISWVRQAPGQGLEWMGW

SEQ ID NO: 134 - protein, 8 aa, synthetic construct
ISAYNGNT

SEQ ID NO: 135 - protein, 38 aa, synthetic construct [sequence omitted]

SEQ ID NO: 136 - protein, 11 aa, synthetic construct
ARWGRWLAHDY

SEQ ID NO: 137 - protein, 11 aa, synthetic construct
WGQGTLVTVSS

SEQ ID NO: 138 - protein, 29 aa, synthetic construct
QIQLVQSGAEVKKPGASVKVSCKASGYTF

SEQ ID NO: 139 - protein, 7 aa, synthetic construct
GYTFTSY

SEQ ID NO: 140 - protein, 10 aa, synthetic construct
GYTFTSYGIS

SEQ ID NO: 141 - protein, 6 aa, synthetic construct
TSYGIS

SEQ ID NO: 142 - protein, 19 aa, synthetic construct
GISWVRQAPGQGLEWMGWI

SEQ ID NO: 143 - protein, 11 aa, synthetic construct
WVRQAPGQGLE

SEQ ID NO: 144 - protein, 6 aa, synthetic construct
SAYNGN

SEQ ID NO: 145 - protein, 10 aa, synthetic construct
WISAYNGNTN

SEQ ID NO: 146 - protein, 13 aa, synthetic construct
WMGWISAYNGNTN

SEQ ID NO: 147 - protein, 41 aa, synthetic construct
TNYAQKLQGRVTMTTDTSTSTAYMELRSLRSDDTAVYYCAR

SEQ ID NO: 148 - protein, 39 aa, synthetic construct
YAQKLQGRVTMTTDTSTSTAYMELRSLRSDDTAVYYCAR

SEQ ID NO: 149 - protein, 37 aa, synthetic construct
YAQKLQGRVTMTTDTSTSTAYMELRSLRSDDTAVYYC

SEQ ID NO: 150 - protein, 10 aa, synthetic construct
ARWGRWLAHD

SEQ ID NO: 151 - protein, 12 aa, synthetic construct
YWGQGTLVTVSS

SEQ ID NO: 152 - protein, 22 aa, synthetic construct
QAVLTQPPSVSVSPGQTASITC

SEQ ID NO: 153 - protein, 28 aa, synthetic construct
QAVLTQPPSVSVSPGQTASITCSGDKLG

SEQ ID NO: 154 - protein, 25 aa, synthetic construct
QAVLTQPPSVSVSPGQTASITCSGD

SEQ ID NO: 155 - protein, 7 aa, synthetic construct
NKNAYWY

SEQ ID NO: 156 - protein, 6 aa, synthetic construct
KLGNKN

SEQ ID NO: 157 - protein, 9 aa, synthetic construct
QQKPGQSPV

SEQ ID NO: 158 - protein, 17 aa, synthetic construct
AYWYQQKPGQSPVLVMY

SEQ ID NO: 159 - protein, 10 aa, synthetic construct
LVMYQSTRRP

SEQ ID NO: 160 - protein, 32 aa, synthetic construct
GIPERFSASNSGNTATLTISGTQAMDEADYYC

SEQ ID NO: 161 - protein, 33 aa, synthetic construct
SGIPERFSASNSGNTATLTISGTQAMDEADYYC

SEQ ID NO: 162 - protein, 37 aa, synthetic construct
TRRPSGIPERFSASNSGNTATLTISGTQAMDEADYYC

SEQ ID NO: 163 - protein, 10 aa, synthetic construct
QAWDSSSGWE

SEQ ID NO: 164 - protein, 10 aa, synthetic construct
FGGGTKLTVL

SEQ ID NO: 165 - protein, 11 aa, synthetic construct
VFGGGTKLTVL

SEQ ID NO: 166 - protein, 11 aa, synthetic construct
QAWLSSSGWEV

SEQ ID NO: 167 - protein, 11 aa, synthetic construct
QAWDSSSGWEV

SEQ ID NO: 168 - protein, 118 aa, synthetic construct
QIQLVQSGAEVKQPGASVSVSCAASGYTFTSYGISWVRQAPGQGLEWMGWISAYNGNTNYAQKLQGRVTMTTDTSTSTAYMELSSLRSDDTAVYYCARWGRWLAHDYWGQGTLVTVSS

SEQ ID NO: 169 - protein, 118 aa, synthetic construct; identical to SEQ ID NO: 168

SEQ ID NO: 170 - protein, 118 aa, synthetic construct; identical to SEQ ID NO: 168

SEQ ID NO: 171 - protein, 108 aa, synthetic construct
QAVLTQPPSVSVSPGQTASITCSGDKLGNKNAYWYQQKPGQSPVLVMYQSTRRPSGIPERFSASNSGNTATLTISGTQAMDEADYYCQAWLSSSGWEVFGGGTKLTVL

SEQ ID NO: 172 - protein, 108 aa, synthetic construct
QAVLTQPPSVSVSPGQTASITCSGDKLGNKNAYWYQQKPGQSPVLVMYQSTRRPSGIPERFSASNSGNTATLTISGTQAEDEADYYCQAWDSSSGWEVFGGGTKLTVL

SEQ ID NO: 173 - protein, 108 aa, synthetic construct; identical to SEQ ID NO: 39

SEQ ID NO: 174 - DNA, 1335 bp, synthetic construct
  source 1..1335: mol_type = other DNA
cagatccagttggtgcaaagtggggctgaggtaaagcagccgggtgcaagtgtgtccgtaagttgtgcagccagtggctacacctttactagttacggaatttcatgggtgcggcaagctcccggtcagggattggaatggatgggatggatttcagcatacaacgggaacacaaattacgctcaaaaattgcagggtcgagttaccatgactacagacacgtctacgtctacagcttacatggaactttccagcctgcggtccgacgacaccgcagtttattattgcgcccgctgggggagatggctcgcgcatgactactgggggcagggcacgctggttaccgtttcctcagcctccaccaagggcccatccgtcttccccctggcgccctgctccaggagcacctccgagagcacagccgccctgggctgcctggtcaaggactacttccccgaaccggtgacggtgtcgtggaactcaggcgccctgaccagcggcgtgcacaccttcccggctgtcctacagtcctcaggactctactccctcagcagcgtggtgaccgtgccctccagcagcttgggcacgaagacctacacctgcaacgtagatcacaagcccagcaacaccaaggtggacaagagagttgagtccaaatatggtcccccatgcccaccctgcccagcacctgagttcgaggggggaccatcagtcttcctgttccccccaaaacccaaggacactctcatgatctcccggacccctgaggtcacgtgcgtggtggtggacgtgagccaggaagaccccgaggtccagttcaactggtacgtggatggcgtggaggtgcataatgccaagacaaagccgcgggaggagcagttcaacagcacgtaccgtgtggtcagcgtcctcaccgtcctgcaccaggactggctgaacggcaaggagtacaagtgcaaggtgtccaacaaaggcctcccgtcctccatcgagaaaaccatctccaaagccaaagggcagccccgagagccacaggtgtacaccctgcccccatcccaggaggagatgaccaagaaccaggtcagcctgacctgcctggtcaaaggcttctaccccagcgacatcgccgtggagtgggagagcaatgggcagccggagaacaactacaagaccacgcctcccgtgctggactccgacggctccttcttcctctacagcaggctaaccgtggacaagagcaggtggcaggaggggaatgtcttctcatgctccgtgatgcatgaggctctgcacaaccactacacacagaagagtctctccctgtctctgggtaaa

SEQ ID NO: 175 - DNA, 1335 bp, synthetic construct; identical to SEQ ID NO: 174
  source 1..1335: mol_type = other DNA

SEQ ID NO: 176 - DNA, 1335 bp, synthetic construct; identical to SEQ ID NO: 174
  source 1..1335: mol_type = other DNA

SEQ ID NO: 177 - DNA, 642 bp, synthetic construct
  source 1..642: mol_type = other DNA
caggcggtgcttactcagcccccaagtgtgtctgtttcccccggtcagactgcgtctataacctgctccggggataaactcggcaacaagaatgcgtactggtaccaacagaagccgggacagagcccagtcttggtcatgtaccaatccacccggagacctagcggcattccagagcgctttagtgcatctaattctggcaatacggcgacgttgaccatcagtggtacacaagcgatggacgaggcagattactactgtcaggcatggctgtcatcatccgggtgggaggtgtttggcggcggaacaaaactcactgtcctaggtcagcccaaggctgcaccaagtgtcactctgttcccgccctcctctgaggagcttcaagccaacaaggccacactggtgtgtctcataagtgacttctacccgggagccgtgacagtggcctggaaggcagatagcagccccgtcaaggcgggagtggagaccaccacaccctccaaacaaagcaacaacaagtacgcggccagcagctatctgagcctgacgcctgagcagtggaagtcccacagaagctacagctgccaggtcacgcatgaagggagcaccgtggagaagacagtggcccctacagaatgttca

SEQ ID NO: 178 - DNA, 642 bp, synthetic construct
  source 1..642: mol_type = other DNA
caggccgtcttgactcaaccaccctccgttagtgtctcccccggccagacggcgagtatcacctgtagtggtgataagctgggcaataagaatgcttactggtaccagcaaaaacccggacagagcccagtgctggtgatgtatcagtctacaagacgacctagcggcatcccagaaaggttttctgccagcaattctggcaatacggcgacgctgactattagtggcacacaagcagaggatgaggcggactattactgccaagcatgggacagtagtagtggttgggaagtcttcgggggcggcactaagctcaccgtcctaggtcagcccaaggctgcaccaagtgtcactctgttcccgccctcctctgaggagcttcaagccaacaaggccacactggtgtgtctcataagtgacttctacccgggagccgtgacagtggcctggaaggcagatagcagccccgtcaaggcgggagtggagaccaccacaccctccaaacaaagcaacaacaagtacgcggccagcagctatctgagcctgacgcctgagcagtggaagtcccacagaagctacagctgccaggtcacgcatgaagggagcaccgtggagaagacagtggcccctacagaatgttca

SEQ ID NO: 179 - DNA, 642 bp, synthetic construct
  source 1..642: mol_type = other DNA
caagctgtattgacacaacctcctagtgtcagtgtaagccctggtcaaactgcctccattacttgctctggcgacaagctcggaaataagaacgcgtactggtaccaacagaagcccggacagtcacctgtgcttgttatgtatcaaagcaccaggagaccttcagggataccagaaaggtttagtgcgtctaattccgggaataccgcgacactgacgataagcggcactcaggctatggacgaagcggattactactgtcaggcatgggattcatcatcaggttgggaagtattcgggggcggtacaaaattgacggtcctaggtcagcccaaggctgcaccaagtgtcactctgttcccgccctcctctgaggagcttcaagccaacaaggccacactggtgtgtctcataagtgacttctacccgggagccgtgacagtggcctggaaggcagatagcagccccgtcaaggcgggagtggagaccaccacaccctccaaacaaagcaacaacaagtacgcggccagcagctatctgagcctgacgcctgagcagtggaagtcccacagaagctacagctgccaggtcacgcatgaagggagcaccgtggagaagacagtggcccctacagaatgttca

SEQ ID NO: 180 - protein, 326 aa, synthetic construct
ASTKGPSVFPLAPCSRSTSESTAALGCLVKDYFPEPVTVSWNSGALTSGVHTFPAVLQSSGLYSLSSVVTVPSSSLGTKTYTCNVDHKPSNTKVDKRVESKYGPPCPPCPAPEFEGGPSVFLFPPKPKDTLMISRTPEVTCVVVDVSQEDPEVQFNWYVDGVEVHNAKTKPREEQFNSTYRVVSVLTVLHQDWLNGKEYKCKVSNKGLPSSIEKTISKAKGQPREPQVYTLPPSQEEMTKNQVSLTCLVKGFYPSDIAVEWESNGQPENNYKTTPPVLDSDGSFFLYSRLTVDKSRWQEGNVFSCSVMHEALHNHYTQKSLSLSLG